European Patent Specification EP 3 507 384 B1, published August 30, 2023. Title: COMPOSITIONS AND METHODS USING A PHARMACOGENOMICS MARKER. Applicant: DENOVO BIOPHARMA LLC LUO, Wen SUN, Hong. Application Not Yet Assigned. The sequence listing filed with the application follows.

SEQUENCE LISTING (28 sequences)

SEQ ID NO: 1 - DNA, 51 bp, Homo sapiens
  misc_feature 26: n = a or g
tggggaatgtcattccatgttaggcntcatgttgaaacatattatttcata

SEQ ID NO: 2 - DNA, 51 bp, Homo sapiens
  misc_feature 26: n = c or t
gaaggaacactttccctaatgcccangaaggaacaaggattctgatagctt

SEQ ID NO: 3 - DNA, 51 bp, Homo sapiens
  misc_feature 26: n = null or a
aaaagcaaaaaaaaaataaaaaaatnaaaaaaaaaaggcaaagagacagaa

SEQ ID NO: 4 - DNA, 51 bp, Homo sapiens
  misc_feature 26: n = g or t
cacccgttaaaaaaaaaaaaaaatcngtcactaattgttccggttactatt

SEQ ID NO: 5 - DNA, 51 bp, Homo sapiens
  misc_feature 26: n = g or t
atagcaataggcaacaaacaaactancaaatatagtgtcaagtaccaaaag

SEQ ID NO: 6 - DNA, 51 bp, Homo sapiens
  misc_feature 26: n = c or t
cattctcatcatagtctgcttctcanttgattcagtattggatgaagatca

SEQ ID NO: 7 - DNA, 51 bp, Homo sapiens
  misc_feature 26: n = c or t
gctctattttataaaagtctattaantttaactgaaatcaaaataactaca

SEQ ID NO: 8 - DNA, 51 bp, Homo sapiens
  misc_feature 26: n = g or t
tgaatttcatccaaagccttttctgnatctatttagataataatgtggttt

SEQ ID NO: 9 - DNA, 51 bp, Homo sapiens
  misc_feature 26: n = g or t
atccaaagccttttctggatctattnagataataatgtggtttttgtcttt

SEQ ID NO: 10 - DNA, 51 bp, Homo sapiens
  misc_feature 26: n = a or c
ctacagaccaagtgaacaacagaggnctgctgaattcattcattgcatttt

SEQ ID NO: 11 - DNA, 51 bp, Homo sapiens
  misc_feature 26: n = a or t
aacttggggcactctgcactactgcntgccagcattttaaaaagtcatcag

SEQ ID NO: 12 - DNA, 51 bp, Homo sapiens
  misc_feature 26: n = a or g
catacaccaagagttttataaataantttatttcaatatgaaggttaaatt

SEQ ID NO: 13 - DNA, 51 bp, Homo sapiens
  misc_feature 26: n = a or t
ttaatcggaatgctccctgctcctcnctttattccctagataaacgtacac

SEQ ID NO: 14 - DNA, 51 bp, Homo sapiens
  misc_feature 26: n = a or g
atatcatttacattagcaacctctanaataaaatatttaggtattagccta

SEQ ID NO: 15 - DNA, 51 bp, Homo sapiens
  misc_feature 26: n = c or t
ctattattttcagaacattgcttaanatgttggttgagtccggcagacaaa

SEQ ID NO: 16 - DNA, 51 bp, Homo sapiens
  misc_feature 26: n = c or t
tttattgaaatacttaaatttactantgtaaatacttttatacttttatat

SEQ ID NO: 17 - DNA, 51 bp, Homo sapiens
  misc_feature 26: n = c or t
gacctaggagctccccaagccagggntgtgacaccgtctttggggatctct

SEQ ID NO: 18 - DNA, 51 bp, Homo sapiens
  misc_feature 26: n = c or t
tccatttaaaattatcacgcttcttnttctctactcgtcaacatccaacac

SEQ ID NO: 19 - DNA, 51 bp, Homo sapiens
  misc_feature 26: n = c or t
cagaaccaagaacttttctgacctcntcctgtttcttcccctaagtgccag

SEQ ID NO: 20 - DNA, 51 bp, Homo sapiens
  misc_feature 26: n = a or g
tcgttcacaattctaccttatgacanggtcagaaacagaacatagtagatg

SEQ ID NO: 21 - DNA, 51 bp, Homo sapiens
  misc_feature 26: n = a or g
attattatcttccatattaaatacangtttcctttgttggggctcagaaaa

SEQ ID NO: 22 - DNA, 51 bp, Homo sapiens
  misc_feature 26: n = c or t
gaaaaatccatcactttcctatatantagcaataaacatgtggaatttgaa

SEQ ID NO: 23 - DNA, 51 bp, Homo sapiens
  misc_feature 26: n = null or a
ggcaacaagagtgaaacttcatctcnaaaaaaaaaaaaaaaaaaagctgaa

SEQ ID NO: 24 - DNA, 51 bp, Homo sapiens
  misc_feature 26: n = c or t
cacaggttgtggtgagccgagatccntccattgtactcattgcattccagc

SEQ ID NO: 25 - DNA, 51 bp, Homo sapiens
  misc_feature 26: n = a or c
gcacaggttgtggtgagccgagatcnttccattgtactcattgcattccag

SEQ ID NO: 26 - DNA, 51 bp, Homo sapiens
  misc_feature 26: n = g or t
aaaaccaaaccaaagactgagaaatnattagaagccactggaagtttttta

SEQ ID NO: 27 - DNA, 51 bp, Homo sapiens
  misc_feature 26: n = a or g
atttatccaaatgcctttccatggcnttcactgagcaaattctggattttt

SEQ ID NO: 28 - DNA, 51 bp, Homo sapiens
  misc_feature 26: n = a or t
tttccatgtagacagaagaatgaggngctaccctagtgtgtcccttaatga